European Patent Specification EP 3 494 975 B1, published July 24, 2024. Title: COMBINED TELOMERASE INHIBITOR AND GEMCITABINE FOR THE TREAMENT OF CANCER. Applicant: Geron Corporation et al. Go, Ning Tressler, Robert J. Application To be Assigned. The sequence listing filed with the application follows.

SEQUENCE LISTING (27 sequences)

SEQ ID NO: 1 - RNA, 554 nt, Homo sapiens
ggguugcggagggugggccugggaggggugguggccauuuuuugucuaacccuaacugagaagggcguaggcgccgugcuuuugcuccccgcgcgcuguuuuucucgcugacuuucagcgggcggaaaagccucggccugccgccuuccaccguucauucuagagcaaacaaaaaaugucagcugcuggcccguucgccucccggggaccugcggcgggucgccugcccagcccccgaaccccgccuggagccgcggucggcccggggcuucuccggaggcacccacugccaccgcgaagaguugggcucugucagccgcgggucucucgggggcgagggcgagguucaccguuucaggccgcaggaagaggaacggagcgagucccgccgcggcgcgauucccugagcugugggacgugcacccaggacucggcucacacaugcaguucgcuuuccuguugguggggggaacgccgaucgugcgcauccgucaccccucgccggcagugggggcuugugaacccccaaaccugacugacugggccagugugcu

SEQ ID NO: 2 - DNA, 20 bp, Artificial Sequence
  Oligonucleotide
acattttttgtttgctctag

SEQ ID NO: 3 - DNA, 30 bp, Artificial Sequence
  Oligonucleotide
gctctagaatgaacggtggaaggcggcagg

SEQ ID NO: 4 - DNA, 14 bp, Artificial Sequence
  Oligonucleotide
gtggaggcggcagg

SEQ ID NO: 5 - DNA, 13 bp, Artificial Sequence
  Oligonucleotide
ggaaggcggcagg

SEQ ID NO: 6 - DNA, 13 bp, Artificial Sequence
  Oligonucleotide
gtggaaggcggca

SEQ ID NO: 7 - DNA, 11 bp, Artificial Sequence
  Oligonucleotide
gtggaaggcgg

SEQ ID NO: 8 - DNA, 13 bp, Artificial Sequence
  Oligonucleotide
cggtggaaggcgg

SEQ ID NO: 9 - DNA, 13 bp, Artificial Sequence
  Oligonucleotide
acggtggaaggcg

SEQ ID NO: 10 - DNA, 16 bp, Artificial Sequence
  Oligonucleotide
aacggtggaaggcggc

SEQ ID NO: 11 - DNA, 18 bp, Artificial Sequence
  Oligonucleotide
atgaacggtggaaggcgg

SEQ ID NO: 12 - DNA, 13 bp, Artificial Sequence
  Oligonucleotide
tagggttagacaa

SEQ ID NO: 13 - DNA, 13 bp, Artificial Sequence
  Oligonucleotide
cagttagggttag

SEQ ID NO: 14 - DNA, 12 bp, Artificial Sequence
  Oligonucleotide
tagggttagaca

SEQ ID NO: 15 - DNA, 11 bp, Artificial Sequence
  Oligonucleotide
tagggttagac

SEQ ID NO: 16 - DNA, 11 bp, Artificial Sequence
  Oligonucleotide
gttagggttag

SEQ ID NO: 17 - DNA, 13 bp, Artificial Sequence
  Oligonucleotide
gttagggttagac

SEQ ID NO: 18 - DNA, 15 bp, Artificial Sequence
  Oligonucleotide
gttagggttagacaa

SEQ ID NO: 19 - DNA, 9 bp, Artificial Sequence
  Oligonucleotide
gggttagac

SEQ ID NO: 20 - DNA, 9 bp, Artificial Sequence
  Oligonucleotide
cagttaggg

SEQ ID NO: 21 - DNA, 12 bp, Artificial Sequence
  Oligonucleotide
cccttctcagtt

SEQ ID NO: 22 - DNA, 12 bp, Artificial Sequence
  Oligonucleotide
cgcccttctcag

SEQ ID NO: 23 - DNA, 13 bp, Artificial Sequence
  Oligonucleotide
taggtgtaagcaa

SEQ ID NO: 24 - DNA, 13 bp, Artificial Sequence
  Oligonucleotide
ttgtctaacccta

SEQ ID NO: 25 - DNA, 11 bp, Artificial Sequence
  Oligonucleotide
gttgagtgtag

SEQ ID NO: 26 - DNA, 6 bp, Artificial Sequence
  Oligonucleotide
ttaggg

SEQ ID NO: 27 - DNA, 10 bp, Artificial Sequence
  Oligonucleotide
tttttttttt